European Patent Application EP 4 567 112 A1, published June 11, 2025. Title: 一种抑制APOC3基因表达的RNA抑制剂及其应用. Applicant: 厦门甘宝利生物医药有限公司. Application CN. The sequence listing filed with the application follows.

SEQUENCE LISTING (86 sequences)

SEQ ID NO: 1 - RNA, 23 nt, synthetic construct
  source 1..23: mol_type = other RNA
  misc_feature 22..23: note = t is thymidine
ttacatgaagcacgccaccaatt

SEQ ID NO: 2 - RNA, 23 nt, synthetic construct
  source 1..23: mol_type = other RNA
  misc_feature 22..23: note = t is thymidine
ttggtggcgtgcttcatgtaatt

SEQ ID NO: 3 - RNA, 23 nt, synthetic construct
  source 1..23: mol_type = other RNA
  misc_feature 22..23: note = t is thymidine
tctcagcttcatgcagggttatt

SEQ ID NO: 4 - RNA, 23 nt, synthetic construct
  source 1..23: mol_type = other RNA
  misc_feature 22..23: note = t is thymidine
taaccctgcatgaagctgagatt

SEQ ID NO: 5 - RNA, 23 nt, synthetic construct
  source 1..23: mol_type = other RNA
  misc_feature 22..23: note = t is thymidine
agactactggagcaccgttaatt

SEQ ID NO: 6 - RNA, 23 nt, synthetic construct
  source 1..23: mol_type = other RNA
  misc_feature 22..23: note = t is thymidine
ttaacggtgctccagtagtcttt

SEQ ID NO: 7 - RNA, 23 nt, synthetic construct
  source 1..23: mol_type = other RNA
  misc_feature 22..23: note = t is thymidine
ccgttaaggacaagttctctgtt

SEQ ID NO: 8 - RNA, 23 nt, synthetic construct
  source 1..23: mol_type = other RNA
  misc_feature 22..23: note = t is thymidine
cagagaacttgtccttaacggtt

SEQ ID NO: 9 - RNA, 23 nt, synthetic construct
  source 1..23: mol_type = other RNA
  misc_feature 22..23: note = t is thymidine
tggctgcctgagacctcaatatt

SEQ ID NO: 10 - RNA, 23 nt, synthetic construct
  source 1..23: mol_type = other RNA
  misc_feature 22..23: note = t is thymidine
tattgaggtctcaggcagccatt

SEQ ID NO: 11 - RNA, 23 nt, synthetic construct
  source 1..23: mol_type = other RNA
  misc_feature 22..23: note = t is thymidine
cctgaggtcagaccaacttcatt

SEQ ID NO: 12 - RNA, 23 nt, synthetic construct
  source 1..23: mol_type = other RNA
  misc_feature 22..23: note = t is thymidine
tgaagttggtctgacctcaggtt

SEQ ID NO: 13 - RNA, 23 nt, synthetic construct
  source 1..23: mol_type = other RNA
  misc_feature 22..23: note = t is thymidine
aagggacagtattctcagtgctt

SEQ ID NO: 14 - RNA, 23 nt, synthetic construct
  source 1..23: mol_type = other RNA
gcactgagaatactgtccctttt

SEQ ID NO: 15 - RNA, 21 nt, synthetic construct
  source 1..21: mol_type = other RNA
gggacagtattctcagtgcta

SEQ ID NO: 16 - RNA, 21 nt, synthetic construct
  source 1..21: mol_type = other RNA
gcactgagaatactgtccctt

SEQ ID NO: 17 - RNA, 21 nt, synthetic construct
  source 1..21: mol_type = other RNA
tagggacagtattctcagtgt

SEQ ID NO: 18 - RNA, 21 nt, synthetic construct
  source 1..21: mol_type = other RNA
acactgagaatactgtcccta

SEQ ID NO: 19 - RNA, 21 nt, synthetic construct
  source 1..21: mol_type = other RNA
gcttaaaagggacagtattca

SEQ ID NO: 20 - RNA, 21 nt, synthetic construct
  source 1..21: mol_type = other RNA
tgaatactgtcccttttaagc

SEQ ID NO: 21 - RNA, 21 nt, synthetic construct
  source 1..21: mol_type = other RNA
aaagggacagtattctcagtg

SEQ ID NO: 22 - RNA, 21 nt, synthetic construct
  source 1..21: mol_type = other RNA
ctgagaatactgtccctttta

SEQ ID NO: 23 - RNA, 21 nt, synthetic construct
  source 1..21: mol_type = other RNA
aagggacagtattctcagtgc

SEQ ID NO: 24 - RNA, 21 nt, synthetic construct
  source 1..21: mol_type = other RNA
actgagaatactgtcccttta

SEQ ID NO: 25 - RNA, 21 nt, synthetic construct
  source 1..21: mol_type = other RNA
gcttaaaagggacagtattca

SEQ ID NO: 26 - RNA, 22 nt, synthetic construct
  source 1..22: mol_type = other RNA
taatactgtcccttttaagcaa

SEQ ID NO: 27 - RNA, 21 nt, synthetic construct
  source 1..21: mol_type = other RNA
gtggctgcctgagacctcaat

SEQ ID NO: 28 - RNA, 21 nt, synthetic construct
  source 1..21: mol_type = other RNA
tgaggtctcaggcagccacgg

SEQ ID NO: 29 - RNA, 21 nt, synthetic construct
  source 1..21: mol_type = other RNA
aagtccacctgcctatccatc

SEQ ID NO: 30 - RNA, 21 nt, synthetic construct
  source 1..21: mol_type = other RNA
tggataggcaggtggacttgg

SEQ ID NO: 31 - RNA, 21 nt, synthetic construct
  source 1..21: mol_type = other RNA
cacctgcctatccatcctgaa

SEQ ID NO: 32 - RNA, 21 nt, synthetic construct
  source 1..21: mol_type = other RNA
caggatggataggcaggtgga

SEQ ID NO: 33 - RNA, 21 nt, synthetic construct
  source 1..21: mol_type = other RNA
gggacagtattctcagtgctt

SEQ ID NO: 34 - RNA, 21 nt, synthetic construct
  source 1..21: mol_type = other RNA
gcactgagaatactgtccctt

SEQ ID NO: 35 - RNA, 21 nt, synthetic construct
  source 1..21: mol_type = other RNA
gacagtattctcagtgctctt

SEQ ID NO: 36 - RNA, 21 nt, synthetic construct
  source 1..21: mol_type = other RNA
gagcactgagaatactgtccc

SEQ ID NO: 37 - RNA, 21 nt, synthetic construct
  source 1..21: mol_type = other RNA
gagcgacagtattctcagtgt

SEQ ID NO: 38 - RNA, 21 nt, synthetic construct
  source 1..21: mol_type = other RNA
acactgagaatactgtcgctc

SEQ ID NO: 39 - RNA, 21 nt, synthetic construct
  source 1..21: mol_type = other RNA
aagcgacagtattctcagtgt

SEQ ID NO: 40 - RNA, 21 nt, synthetic construct
  source 1..21: mol_type = other RNA
acactgagaatactgtcgctt

SEQ ID NO: 41 - RNA, 21 nt, synthetic construct
  source 1..21: mol_type = other RNA
aagggacagtattctcagtga

SEQ ID NO: 42 - RNA, 21 nt, synthetic construct
  source 1..21: mol_type = other RNA
tcactgagaatactgtccctt

SEQ ID NO: 43 - RNA, 21 nt, synthetic construct
  source 1..21: mol_type = other RNA
  misc_feature 1..21: note = 2' -OH of the nucleotides at positions 9, 10, 11 from the 5' end of the sense strand is replaced by fluorine, 2' -OH of the remaining nucleotides in the sense strand is replaced by methoxy group, and there are two consecutive phosphorothioate linkages between 3 adjacent nucleotides at the 5' and 3' ends of the sense strand
ttacatgaagcacgccaccaa

SEQ ID NO: 44 - RNA, 21 nt, synthetic construct
  source 1..21: mol_type = other RNA
  misc_feature 1..21: note = 2' -OH of the nucleotides at positions 2, 4, 6, 8, 14, 16 from the 5' end of the antisense strand is replaced by fluorine, 2' -OH of the remaining nucleotides in the antisense strand is replaced by methoxy group, and there are two consecutive phosphorothioate linkages between 3 adjacent nucleotides at the 5' and 3' ends of the antisense strand
ttggtggcgtgcttcatgtaa

SEQ ID NO: 45 - RNA, 21 nt, synthetic construct
  source 1..21: mol_type = other RNA
  misc_feature 1..21: note = 2' -OH of the nucleotides at positions 9, 10, 11 from the 5' end of the sense strand is replaced by fluorine, 2' -OH of the remaining nucleotides in the sense strand is replaced by methoxy group, and there are two consecutive phosphorothioate linkages between 3 adjacent nucleotides at the 5' and 3' ends of the sense strand
tctcagcttcatgcagggtta

SEQ ID NO: 46 - RNA, 21 nt, synthetic construct
  source 1..21: mol_type = other RNA
  misc_feature 1..21: note = 2' -OH of the nucleotides at positions 2, 4, 6, 8, 14, 16 from the 5' end of the antisense strand is replaced by fluorine, 2' -OH of the remaining nucleotides in the antisense strand is replaced by methoxy group, and there are two consecutive phosphorothioate linkages between 3 adjacent nucleotides at the 5' and 3' ends of the antisense strand
taaccctgcatgaagctgaga

SEQ ID NO: 47 - RNA, 21 nt, synthetic construct
  source 1..21: mol_type = other RNA
  misc_feature 1..21: note = 2' -OH of the nucleotides at positions 9, 10, 11 from the 5' end of the sense strand is replaced by fluorine, 2' -OH of the remaining nucleotides in the sense strand is replaced by methoxy group, and there are two consecutive phosphorothioate linkages between 3 adjacent nucleotides at the 5' and 3' ends of the sense strand
agactactggagcaccgttaa

SEQ ID NO: 48 - RNA, 21 nt, synthetic construct
  source 1..21: mol_type = other RNA
  misc_feature 1..21: note = 2' -OH of the nucleotides at positions 2, 4, 6, 8, 14, 16 from the 5' end of the antisense strand is replaced by fluorine, 2' -OH of the remaining nucleotides in the antisense strand is replaced by methoxy group, and there are two consecutive phosphorothioate linkages between 3 adjacent nucleotides at the 5' and 3' ends of the antisense strand
ttaacggtgctccagtagtct

SEQ ID NO: 49 - RNA, 21 nt, synthetic construct
  source 1..21: mol_type = other RNA
  misc_feature 1..21: note = 2' -OH of the nucleotides at positions 9, 10, 11 from the 5' end of the sense strand is replaced by fluorine, 2' -OH of the remaining nucleotides in the sense strand is replaced by methoxy group, and there are two consecutive phosphorothioate linkages between 3 adjacent nucleotides at the 5' and 3' ends of the sense strand
ccgttaaggacaagttctctg

SEQ ID NO: 50 - RNA, 21 nt, synthetic construct
  source 1..21: mol_type = other RNA
  misc_feature 1..21: note = 2' -OH of the nucleotides at positions 2, 4, 6, 8, 14, 16 from the 5' end of the antisense strand is replaced by fluorine, 2' -OH of the remaining nucleotides in the antisense strand is replaced by methoxy group, and there are two consecutive phosphorothioate linkages between 3 adjacent nucleotides at the 5' and 3' ends of the antisense strand
cagagaacttgtccttaacgg

SEQ ID NO: 51 - RNA, 21 nt, synthetic construct
  source 1..21: mol_type = other RNA
  misc_feature 1..21: note = 2' -OH of the nucleotides at positions 9, 10, 11 from the 5' end of the sense strand is replaced by fluorine, 2' -OH of the remaining nucleotides in the sense strand is replaced by methoxy group, and there are two consecutive phosphorothioate linkages between 3 adjacent nucleotides at the 5' and 3' ends of the sense strand
tggctgcctgagacctcaata

SEQ ID NO: 52 - RNA, 21 nt, synthetic construct
  source 1..21: mol_type = other RNA
  misc_feature 1..21: note = 2' -OH of the nucleotides at positions 2, 4, 6, 8, 14, 16 from the 5' end of the antisense strand is replaced by fluorine, 2' -OH of the remaining nucleotides in the antisense strand is replaced by methoxy group, and there are two consecutive phosphorothioate linkages between 3 adjacent nucleotides at the 5' and 3' ends of the antisense strand
tattgaggtctcaggcagcca

SEQ ID NO: 53 - RNA, 21 nt, synthetic construct
  source 1..21: mol_type = other RNA
  misc_feature 1..21: note = 2' -OH of the nucleotides at positions 9, 10, 11 from the 5' end of the sense strand is replaced by fluorine, 2' -OH of the remaining nucleotides in the sense strand is replaced by methoxy group, and there are two consecutive phosphorothioate linkages between 3 adjacent nucleotides at the 5' and 3' ends of the sense strand
cctgaggtcagaccaacttca

SEQ ID NO: 54 - RNA, 21 nt, synthetic construct
  source 1..21: mol_type = other RNA
  misc_feature 1..21: note = 2' -OH of the nucleotides at positions 2, 4, 6, 8, 14, 16 from the 5' end of the antisense strand is replaced by fluorine, 2' -OH of the remaining nucleotides in the antisense strand is replaced by methoxy group, and there are two consecutive phosphorothioate linkages between 3 adjacent nucleotides at the 5' and 3' ends of the antisense strand
tgaagttggtctgacctcagg

SEQ ID NO: 55 - RNA, 21 nt, synthetic construct
  source 1..21: mol_type = other RNA
  misc_feature 1..21: note = 2' -OH of the nucleotides at positions 9, 10, 11 from the 5' end of the sense strand is replaced by fluorine, 2' -OH of the remaining nucleotides in the sense strand is replaced by methoxy group, and there are two consecutive phosphorothioate linkages between 3 adjacent nucleotides at the 5' and 3' ends of the sense strand
aagggacagtattctcagtgc

SEQ ID NO: 56 - RNA, 23 nt, synthetic construct
  source 1..23: mol_type = other RNA
  misc_feature 1..23: note = 2' -OH of the nucleotides at positions 2, 4, 6, 8, 14, 16 from the 5' end of the antisense strand is replaced by fluorine, 2' -OH of the remaining nucleotides in the antisense strand is replaced by methoxy group, and there are two consecutive phosphorothioate linkages between 3 adjacent nucleotides at the 5' and 3' ends of the antisense strand
gcactgagaatactgtccctttt

SEQ ID NO: 57 - RNA, 21 nt, synthetic construct
  source 1..21: mol_type = other RNA
  misc_feature 1..21: note = 2' -OH of the nucleotides at positions 5, 7, 8, 9 from the 5' end of the sense strand is replaced by fluorine, 2' -OH of the remaining nucleotides in the sense strand is replaced by methoxy group, and there are two consecutive phosphorothioate linkages between 3 adjacent nucleotides at the 5' and 3' ends of the sense strand
gggacagtattctcagtgcta

SEQ ID NO: 58 - RNA, 21 nt, synthetic construct
  source 1..21: mol_type = other RNA
  misc_feature 1..21: note = 2' -OH of the nucleotides at positions 7, 12, 14 from the 5' end of the antisense strand is replaced by fluorine, 2' -OH of the remaining nucleotides in the antisense strand is replaced by methoxy group, and there are two consecutive phosphorothioate linkages between 3 adjacent nucleotides at the 5' and 3' ends of the antisense strand
gcactgagaatactgtccctt

SEQ ID NO: 59 - RNA, 21 nt, synthetic construct
  source 1..21: mol_type = other RNA
  misc_feature 1..21: note = 2' -OH of the nucleotides at positions 5, 7, 8, 9 from the 5' end of the sense strand is replaced by fluorine, 2' -OH of the remaining nucleotides in the sense strand is replaced by methoxy group, and there are two consecutive phosphorothioate linkages between 3 adjacent nucleotides at the 5' and 3' ends of the sense strand
  misc_feature 15: note = T is thymidine
tagggacagtattctcagtgt

SEQ ID NO: 60 - RNA, 21 nt, synthetic construct
  source 1..21: mol_type = other RNA
  misc_feature 1..21: note = 2' -OH of the nucleotides at positions 7, 12, 14 from the 5' end of the antisense strand is replaced by fluorine, 2' -OH of the remaining nucleotides in the antisense strand is replaced by methoxy group, and there are two consecutive phosphorothioate linkages between 3 adjacent nucleotides at the 5' and 3' ends of the antisense strand
acactgagaatactgtcccta

SEQ ID NO: 61 - RNA, 21 nt, synthetic construct
  source 1..21: mol_type = other RNA
  misc_feature 1..21: note = 2' -OH of the nucleotides at positions 9, 10, 11 from the 5' end of the sense strand is replaced by fluorine, 2' -OH of the remaining nucleotides in the sense strand is replaced by methoxy group, and there are two consecutive phosphorothioate linkages between 3 adjacent nucleotides at the 5' and 3' ends of the sense strand
gcttaaaagggacagtattca

SEQ ID NO: 62 - RNA, 21 nt, synthetic construct
  source 1..21: mol_type = other RNA
  misc_feature 1..21: note = 2' -OH of the nucleotides at positions 2, 4, 6, 8, 10, 12, 14, 16, 18 from the 5' end of the antisense strand is replaced by fluorine, 2' -OH of the remaining nucleotides in the antisense strand is replaced by methoxy group, and there are two consecutive phosphorothioate linkages between 3 adjacent nucleotides at the 5' and 3' ends of the antisense strand
tgaatactgtcccttttaagc

SEQ ID NO: 63 - RNA, 21 nt, synthetic construct
  source 1..21: mol_type = other RNA
  misc_feature 1..21: note = 2' -OH of the nucleotides at positions 5, 7, 8, 9 from the 5' end of the sense strand is replaced by fluorine, 2' -OH of the remaining nucleotides in the sense strand is replaced by methoxy group, and there are two consecutive phosphorothioate linkages between 3 adjacent nucleotides at the 5' and 3' ends of the sense strand
aaagggacagtattctcagtg

SEQ ID NO: 64 - RNA, 21 nt, synthetic construct
  source 1..21: mol_type = other RNA
  misc_feature 1..21: note = 2' -OH of the nucleotides at positions 2, 4, 6, 8, 14, 16 from the 5' end of the antisense strand is replaced by fluorine, 2' -OH of the remaining nucleotides in the antisense strand is replaced by methoxy group, and there are two consecutive phosphorothioate linkages between 3 adjacent nucleotides at the 5' and 3' ends of the antisense strand
ctgagaatactgtccctttta

SEQ ID NO: 65 - RNA, 21 nt, synthetic construct
  source 1..21: mol_type = other RNA
  misc_feature 1..21: note = 2' -OH of the nucleotides at positions 5, 7, 8, 9 from the 5' end of the sense strand is replaced by fluorine, 2' -OH of the remaining nucleotides in the sense strand is replaced by methoxy group, and there are two consecutive phosphorothioate linkages between 3 adjacent nucleotides at the 5' and 3' ends of the sense strand
aagggacagtattctcagtgc

SEQ ID NO: 66 - RNA, 21 nt, synthetic construct
  source 1..21: mol_type = other RNA
  misc_feature 1..21: note = 2' -OH of the nucleotides at positions 7, 12, 14 from the 5' end of the antisense strand is replaced by fluorine, 2' -OH of the remaining nucleotides in the antisense strand is replaced by methoxy group, and there are two consecutive phosphorothioate linkages between 3 adjacent nucleotides at the 5' and 3' ends of the antisense strand
actgagaatactgtcccttta

SEQ ID NO: 67 - RNA, 21 nt, synthetic construct
  source 1..21: mol_type = other RNA
  misc_feature 1..21: note = 2' -OH of the nucleotides at positions 9, 10, 11 from the 5' end of the sense strand is replaced by fluorine, 2' -OH of the remaining nucleotides in the sense strand is replaced by methoxy group, and there are two consecutive phosphorothioate linkages between 3 adjacent nucleotides at the 5' and 3' ends of the sense strand
gcttaaaagggacagtattca

SEQ ID NO: 68 - RNA, 22 nt, synthetic construct
  source 1..22: mol_type = other RNA
  misc_feature 1..21: note = 2' -OH of the nucleotides at positions 3, 5, 7, 9, 11, 13, 15, 17 from the 5' end of the antisense strand is replaced by fluorine, 2' -OH of the remaining nucleotides in the antisense strand is replaced by methoxy group, and there are two consecutive phosphorothioate linkages between 3 adjacent nucleotides at the 5' and 3' ends of the antisense strand
taatactgtcccttttaagcaa

SEQ ID NO: 69 - RNA, 21 nt, synthetic construct
  source 1..21: mol_type = other RNA
  misc_feature 1..21: note = 2' -OH of the nucleotides at positions 9, 10, 11 from the 5' end of the sense strand is replaced by fluorine, 2' -OH of the remaining nucleotides in the sense strand is replaced by methoxy group, and there are two consecutive phosphorothioate linkages between 3 adjacent nucleotides at the 5' and 3' ends of the sense strand
gtggctgcctgagacctcaat

SEQ ID NO: 70 - RNA, 21 nt, synthetic construct
  source 1..21: mol_type = other RNA
  misc_feature 1..21: note = 2' -OH of the nucleotides at positions 2, 4, 6, 8, 14, 16, 18, 20 from the 5' end of the antisense strand is replaced by fluorine, 2' -OH of the remaining nucleotides in the antisense strand is replaced by methoxy group, and there are two consecutive phosphorothioate linkages between 3 adjacent nucleotides at the 5' and 3' ends of the antisense strand
tgaggtctcaggcagccacgg

SEQ ID NO: 71 - RNA, 21 nt, synthetic construct
  source 1..21: mol_type = other RNA
  misc_feature 1..21: note = 2' -OH of the nucleotides at positions 9, 10, 11 from the 5' end of the sense strand is replaced by fluorine, 2' -OH of the remaining nucleotides in the sense strand is replaced by methoxy group, and there are two consecutive phosphorothioate linkages between 3 adjacent nucleotides at the 5' and 3' ends of the sense strand
aagtccacctgcctatccatc

SEQ ID NO: 72 - RNA, 21 nt, synthetic construct
  source 1..21: mol_type = other RNA
  misc_feature 1..21: note = 2' -OH of the nucleotides at positions 2, 4, 6, 8, 14, 16, 18, 20 from the 5' end of the antisense strand is replaced by fluorine, 2' -OH of the remaining nucleotides in the antisense strand is replaced by methoxy group, and there are two consecutive phosphorothioate linkages between 3 adjacent nucleotides at the 5' and 3' ends of the antisense strand
tggataggcaggtggacttgg

SEQ ID NO: 73 - RNA, 21 nt, synthetic construct
  source 1..21: mol_type = other RNA
  misc_feature 1..21: note = 2' -OH of the nucleotides at positions 9, 10, 11 from the 5' end of the sense strand is replaced by fluorine, 2' -OH of the remaining nucleotides in the sense strand is replaced by methoxy group, and there are two consecutive phosphorothioate linkages between 3 adjacent nucleotides at the 5' and 3' ends of the sense strand
cacctgcctatccatcctgaa

SEQ ID NO: 74 - RNA, 21 nt, synthetic construct
  source 1..21: mol_type = other RNA
  misc_feature 1..21: note = 2' -OH of the nucleotides at positions 2, 4, 6, 8, 14, 16, 18, 20 from the 5' end of the antisense strand is replaced by fluorine, 2' -OH of the remaining nucleotides in the antisense strand is replaced by methoxy group, and there are two consecutive phosphorothioate linkages between 3 adjacent nucleotides at the 5' and 3' ends of the antisense strand
caggatggataggcaggtgga

SEQ ID NO: 75 - RNA, 21 nt, synthetic construct
  source 1..21: mol_type = other RNA
  misc_feature 1..21: note = 2' -OH of the nucleotides at positions 9, 10, 11 from the 5' end of the sense strand is replaced by fluorine, 2' -OH of the remaining nucleotides in the sense strand is replaced by methoxy group, and there are two consecutive phosphorothioate linkages between 3 adjacent nucleotides at the 5' and 3' ends of the sense strand
gggacagtattctcagtgctt

SEQ ID NO: 76 - RNA, 21 nt, synthetic construct
  source 1..21: mol_type = other RNA
  misc_feature 1..21: note = 2' -OH of the nucleotides at positions 2, 4, 6, 8, 14, 16, 18, 20 from the 5' end of the antisense strand is replaced by fluorine, 2' -OH of the remaining nucleotides in the antisense strand is replaced by methoxy group, and there are two consecutive phosphorothioate linkages between 3 adjacent nucleotides at the 5' and 3' ends of the antisense strand
gcactgagaatactgtccctt

SEQ ID NO: 77 - RNA, 21 nt, synthetic construct
  source 1..21: mol_type = other RNA
  misc_feature 1..21: note = 2' -OH of the nucleotides at positions 9, 10, 11 from the 5' end of the sense strand is replaced by fluorine, 2' -OH of the remaining nucleotides in the sense strand is replaced by methoxy group, and there are two consecutive phosphorothioate linkages between 3 adjacent nucleotides at the 5' and 3' ends of the sense strand
gacagtattctcagtgctctt

SEQ ID NO: 78 - RNA, 21 nt, synthetic construct
  source 1..21: mol_type = other RNA
  misc_feature 1..21: note = 2' -OH of the nucleotides at positions 2, 4, 6, 8, 14, 16, 18, 20 from the 5' end of the antisense strand is replaced by fluorine, 2' -OH of the remaining nucleotides in the antisense strand is replaced by methoxy group, and there are two consecutive phosphorothioate linkages between 3 adjacent nucleotides at the 5' and 3' ends of the antisense strand
gagcactgagaatactgtccc

SEQ ID NO: 79 - RNA, 21 nt, synthetic construct
  source 1..21: mol_type = other RNA
  misc_feature 1..21: note = 2' -OH of the nucleotides at positions 9, 10, 11 from the 5' end of the sense strand is replaced by fluorine, 2' -OH of the remaining nucleotides in the sense strand is replaced by methoxy group, and there are two consecutive phosphorothioate linkages between 3 adjacent nucleotides at the 5' and 3' ends of the sense strand
gagcgacagtattctcagtgt

SEQ ID NO: 80 - RNA, 21 nt, synthetic construct
  source 1..21: mol_type = other RNA
  misc_feature 1..21: note = 2' -OH of the nucleotides at positions 2, 4, 6, 8, 14, 16, 18, 20 from the 5' end of the antisense strand is replaced by fluorine, 2' -OH of the remaining nucleotides in the antisense strand is replaced by methoxy group, and there are two consecutive phosphorothioate linkages between 3 adjacent nucleotides at the 5' and 3' ends of the antisense strand
acactgagaatactgtcgctc

SEQ ID NO: 81 - RNA, 21 nt, synthetic construct
  source 1..21: mol_type = other RNA
  misc_feature 1..21: note = 2' -OH of the nucleotides at positions 7, 9, 10, 11 from the 5' end of the sense strand is replaced by fluorine, 2' -OH of the remaining nucleotides in the sense strand is replaced by methoxy group, and there are two consecutive phosphorothioate linkages between 3 adjacent nucleotides at the 5' and 3' ends of the sense strand
gagcgacagtattctcagtgt

SEQ ID NO: 82 - RNA, 21 nt, synthetic construct
  source 1..21: mol_type = other RNA
  misc_feature 1..21: note = 2' -OH of the nucleotides at positions 2, 4, 6, 8, 10, 14, 16, 18 from the 5' end of the antisense strand is replaced by fluorine, 2' -OH of the remaining nucleotides in the antisense strand is replaced by methoxy group, and there are two consecutive phosphorothioate linkages between 3 adjacent nucleotides at the 5' and 3' ends of the antisense strand
acactgagaatactgtcgctc

SEQ ID NO: 83 - RNA, 21 nt, synthetic construct
  source 1..21: mol_type = other RNA
  misc_feature 1..21: note = 2' -OH of the nucleotides at positions 9, 10, 11 from the 5' end of the sense strand is replaced by fluorine, 2' -OH of the remaining nucleotides in the sense strand is replaced by methoxy group, and there are two consecutive phosphorothioate linkages between 3 adjacent nucleotides at the 5' and 3' ends of the sense strand
aagcgacagtattctcagtgt

SEQ ID NO: 84 - RNA, 21 nt, synthetic construct
  source 1..21: mol_type = other RNA
  misc_feature 1..21: note = 2' -OH of the nucleotides at positions 2, 4, 6, 8, 14, 16, 18, 20 from the 5' end of the antisense strand is replaced by fluorine, 2' -OH of the remaining nucleotides in the antisense strand is replaced by methoxy group, and there are two consecutive phosphorothioate linkages between 3 adjacent nucleotides at the 5' and 3' ends of the antisense strand
acactgagaatactgtcgctt

SEQ ID NO: 85 - RNA, 21 nt, synthetic construct
  source 1..21: mol_type = other RNA
  misc_feature 1..21: note = 2' -OH of the nucleotides at positions 5, 7, 8, 9 from the 5' end of the sense strand is replaced by fluorine, 2' -OH of the remaining nucleotides in the sense strand is replaced by methoxy group, and there are two consecutive phosphorothioate linkages between 3 adjacent nucleotides at the 5' and 3' ends of the sense strand
aagggacagtattctcagtga

SEQ ID NO: 86 - RNA, 21 nt, synthetic construct
  source 1..21: mol_type = other RNA
  misc_feature 1..21: note = 2' -OH of the nucleotides at positions 7, 12, 14 from the 5' end of the antisense strand is replaced by fluorine, 2' -OH of the remaining nucleotides in the antisense strand is replaced by methoxy group, and there are two consecutive phosphorothioate linkages between 3 adjacent nucleotides at the 5' and 3' ends of the antisense strand
tcactgagaatactgtccctt